European Patent Application EP 4 144 361 A1, published March 8, 2023. Title: A pharmaceutical composition for preventing or treating mucositis induced by radiotherapy, cheomotherapy, or a combination thereof, compriging a GLP-2 derivative or a long-acting conjugate thereof. Applicant: HANMI PHARM. CO., LTD. The sequence listing filed with the application follows.

SEQUENCE LISTING (32 sequences)

SEQ ID NO: 1 - protein, 33 aa, Homo sapiens
HADGSFSDEMNTILDNLAARDFINWLIQTKITD

SEQ ID NO: 2 - protein, 34 aa, Artificial Sequence
  GLP-2 derivative
  MISC_FEATURE (1): Xaa is imidazoacetyldeshistidine
XGDGSFSDEMNTILDNLAARDFINWLIQTKITDC

SEQ ID NO: 3 - protein, 34 aa, Artificial Sequence
  GLP-2 derivative
  MISC_FEATURE (1): Xaa is imidazoacetyldeshistidine
XGDGSFSDEMNTILDNLAARDFINWLIQTKITDK

SEQ ID NO: 4 - protein, 34 aa, Artificial Sequence
  GLP-2 derivative
  MISC_FEATURE (1): Xaa is imidazoacetyldeshistidine
XGDGSFSDEMNTILDNLAARDFINWLIQTRITDK

SEQ ID NO: 5 - protein, 34 aa, Artificial Sequence
  GLP-2 derivative
  MISC_FEATURE (1): Xaa is imidazoacetyldeshistidine
  MISC_FEATURE (34): Xaa is 6-azidolysine
XGDGSFSDEMNTILDNLAARDFINWLIQTKITDX

SEQ ID NO: 6 - protein, 34 aa, Artificial Sequence
  GLP-2 derivative
  MISC_FEATURE (1): Xaa is imidazoacetyldeshistidine
XGDGSFSDEMNTILDNLAARDFINWLIQTRITDC

SEQ ID NO: 7 - protein, 34 aa, Artificial Sequence
  GLP-2 derivative
  MISC_FEATURE (1): Xaa is imidazoacetyldeshistidine
  MISC_FEATURE (2): Xaa is Aib(2-aminoisobutyric acid)
XXDGSFSDEMNTILDNLAARDFINWLIQTKITDC

SEQ ID NO: 8 - protein, 34 aa, Artificial Sequence
  GLP-2 derivative
  MISC_FEATURE (2): Xaa is Aib(2-aminoisobutyric acid)
HXDGSFSDEMNTILDNLAARDFINWLIQTKITDC

SEQ ID NO: 9 - protein, 34 aa, Artificial Sequence
  GLP-2 derivative
  MISC_FEATURE (1): Xaa = Histidine, imidazoacetyldeshistidine, desaminohistidine, beta-hydroxyimidazopropionyldeshistidine, N-dimethylhistidine, or beta-carboxyimidazopropionyldeshistidine
  MISC_FEATURE (2): Xaa is Alanine, Glycine, or Aib(2-aminoisobutyric acid)
  MISC_FEATURE (30): Xaa is Lysine, or Arginine
  MISC_FEATURE (34): Xaa is absent, Lysine, Arginine, Glutamine, Histidine, 6-azidolysine, or Cysteine
XXDGSFSDEMNTILDNLAARDFINWLIQTXITDX

SEQ ID NO: 10 - protein, 34 aa, Artificial Sequence; identical to SEQ ID NO: 9
  GLP-2 derivative
  MISC_FEATURE (1): Xaa = Histidine, imidazoacetyldeshistidine, desaminohistidine, beta-hydroxyimidazopropionyldeshistidine, N-dimethylhistidine, or beta-carboxyimidazopropionyldeshistidine
  MISC_FEATURE (2): Xaa is Alanine, Glycine, or Aib(2-aminoisobutyric acid)
  MISC_FEATURE (30): Xaa is Lysine, or Arginine
  MISC_FEATURE (34): Xaa = any one or more amino acid or any one or more amino acid which is modified

SEQ ID NO: 11 - protein, 12 aa, HOMO SAPIENS
ESKYGPPCPSCP

SEQ ID NO: 12 - protein, 11 aa, Artificial Sequence
  Variant of hinge region
ESKYGPPPSCP

SEQ ID NO: 13 - protein, 11 aa, Artificial Sequence
  Variant of hinge region
ESKYGPPCPSP

SEQ ID NO: 14 - protein, 10 aa, Artificial Sequence
  Variant of hinge region
ESKYGPPCPS

SEQ ID NO: 15 - protein, 10 aa, Artificial Sequence
  Variant of hinge region
ESKYGPPCPP

SEQ ID NO: 16 - protein, 8 aa, Artificial Sequence
  Variant of hinge region
KYGPPCPS

SEQ ID NO: 17 - protein, 8 aa, Artificial Sequence
  Variant of hinge region
ESKYGPPC

SEQ ID NO: 18 - protein, 7 aa, Artificial Sequence
  Variant of hinge region
EKYGPPC

SEQ ID NO: 19 - protein, 6 aa, Artificial Sequence
  Variant of hinge region
ESPSCP

SEQ ID NO: 20 - protein, 5 aa, Artificial Sequence
  Variant of hinge region
EPSCP

SEQ ID NO: 21 - protein, 4 aa, Artificial Sequence
  Variant of hinge region
PSCP

SEQ ID NO: 22 - protein, 10 aa, Artificial Sequence
  Variant of hinge region
ESKYGPPSCP

SEQ ID NO: 23 - protein, 9 aa, Artificial Sequence
  Variant of hinge region
KYGPPPSCP

SEQ ID NO: 24 - protein, 9 aa, Artificial Sequence
  Variant of hinge region
ESKYGPSCP

SEQ ID NO: 25 - protein, 8 aa, Artificial Sequence
  Variant of hinge region
ESKYGPPC

SEQ ID NO: 26 - protein, 7 aa, Artificial Sequence
  Variant of hinge region
KYGPPCP

SEQ ID NO: 27 - protein, 7 aa, Artificial Sequence
  Variant of hinge region
ESKPSCP

SEQ ID NO: 28 - protein, 6 aa, Artificial Sequence
  Variant of hinge region
ESPSCP

SEQ ID NO: 29 - protein, 4 aa, Artificial Sequence
  Variant of hinge region
EPSC

SEQ ID NO: 30 - protein, 3 aa, Artificial Sequence
  Variant of hinge region
SCP

SEQ ID NO: 31 - protein, 221 aa, homo sapiens
PSCPAPEFLGGPSVFLFPPKPKDTLMISRTPEVTCVVVDVSQEDPEVQFNWYVDGVEVHNAKTKPREEQFNSTYRVVSVLTVLHQDWLNGKEYKCKVSNKGLPSSIEKTISKAKGQPREPQVYTLPPSQEEMTKNQVSLTCLVKGFYPSDIAVEWESNGQPENNYKTTPPVLDSDGSFFLYSRLTVDKSRWQEGNVFSCSVMHEALHNHYTQKSLSLSLGK

SEQ ID NO: 32 - protein, 442 aa, Homo sapiens
  Human Immunoglobulin G4 Fc Fragment (homodimer)
  MISC_FEATURE (1)..(221): Amino acids at position 1 to 221 form one monomer.
  MISC_FEATURE (222)..(442): Amino acids at position 222 to 442 form one monomer.
  DISULFID (3)..(224): Amino acids at position 3 and position 224 form an inter-disulfide bond
  DISULFID (35)..(95): Amino acids at position 35 and position 95 form an intra-chain disulfide bond.
  DISULFID (141)..(199): Amino acids at position 141 and position 199 form an intra-chain disulfide bond.
  DISULFID (256)..(316): Amino acids at position 256 and position 316 form an intra-chain disulfide bond.
  DISULFID (362)..(420): Amino acids at position 362 and position 420 form an intra-chain disulfide bond
PSCPAPEFLGGPSVFLFPPKPKDTLMISRTPEVTCVVVDVSQEDPEVQFNWYVDGVEVHNAKTKPREEQFNSTYRVVSVLTVLHQDWLNGKEYKCKVSNKGLPSSIEKTISKAKGQPREPQVYTLPPSQEEMTKNQVSLTCLVKGFYPSDIAVEWESNGQPENNYKTTPPVLDSDGSFFLYSRLTVDKSRWQEGNVFSCSVMHEALHNHYTQKSLSLSLGKPSCPAPEFLGGPSVFLFPPKPKDTLMISRTPEVTCVVVDVSQEDPEVQFNWYVDGVEVHNAKTKPREEQFNSTYRVVSVLTVLHQDWLNGKEYKCKVSNKGLPSSIEKTISKAKGQPREPQVYTLPPSQEEMTKNQVSLTCLVKGFYPSDIAVEWESNGQPENNYKTTPPVLDSDGSFFLYSRLTVDKSRWQEGNVFSCSVMHEALHNHYTQKSLSLSLGK